European Patent Application EP 4 563 163 A1, published June 4, 2025. Title: 抗体药物偶联物及其应用. Applicant: 明慧医药（杭州）有限公司. The sequence listing filed with the application follows.

SEQUENCE LISTING (20 sequences)

SEQ ID NO: 1 - protein, 449 aa, synthetic construct
EVQLVESGGGLVQPGGSLRLSCAASGFTFSSYAMSWVRQAPGKGLELVAAINSNGGSTYYADSVKGRFTISRDNAKNTLYLQMSSLRAEDTAVYYCTRNEEFRRGLAYWGQGTLVTVSSASTKGPSVFPLAPSSKSTSGGTAALGCLVKDYFPEPVTVSWNSGALTSGVHTFPAVLQSSGLYSLSSVVTVPSSSLGTQTYICNVNHKPSNTKVDKKVEPKSCDKTHTCPPCPAPELLGGPSVFLFPPKPKDTLMISRTPEVTCVVVDVSHEDPEVKFNWYVDGVEVHNAKTKPREEQYNSTYRVVSVLTVLHQDWLNGKEYKCKVSNKALPAPIEKTISKAKGQPREPQVYTLPPSRDELTKNQVSLTCLVKGFYPSDIAVEWESNGQPENNYKTTPPVLDSDGSFFLYSKLTVDKSRWQQGNVFSCSVMHEALHNHYTQKSLSLSPGK

SEQ ID NO: 2 - protein, 215 aa, synthetic construct
DIQMTQSPSSLSASVGDRVTITCRASENIYSNLAWYQQKPGKAPKLLIYAASNLQSGVPSRFSGSGSGTDYTLTISSLQPEDFATYYCQHFWGTPPWTFGQGTKLEIKRTVAAPSVFIFPPSDEQLKSGTASVVCLLNNFYPREAKVQWKVDNALQSGNSQESVTEQDSKDSTYSLSSTLTLSKADYEKHKVYACEVTHQGLSSPVTKSFNRGEC

SEQ ID NO: 3 - protein, 452 aa, synthetic construct
QVQLVQSGAEVKKPGSSVKVSCKASGYTFTNYVMHWVRQAPGQGLEWMGYINPYNDDVKYNEKFKGRVTITADESTSTAYMELSSLRSEDTAVYYCARWGYYGSPLYYFDYWGQGTLVTVSSASTKGPSVFPLAPSSKSTSGGTAALGCLVKDYFPEPVTVSWNSGALTSGVHTFPAVLQSSGLYSLSSVVTVPSSSLGTQTYICNVNHKPSNTKVDKRVEPKSCDKTHTCPPCPAPELLGGPSVFLFPPKPKDTLMISRTPEVTCVVVDVSHEDPEVKFNWYVDGVEVHNAKTKPREEQYNSTYRVVSVLTVLHQDWLNGKEYKCKVSNKALPAPIEKTISKAKGQPREPQVYTLPPSREEMTKNQVSLTCLVKGFYPSDIAVEWESNGQPENNYKTTPPVLDSDGSFFLYSKLTVDKSRWQQGNVFSCSVMHEALHNHYTQKSLSLSPGK

SEQ ID NO: 4 - protein, 213 aa, synthetic construct
EIVLTQSPATLSLSPGERATLSCRASSRLIYMHWYQQKPGQAPRPLIYATSNLASGIPARFSGSGSGTDFTLTISSLEPEDFAVYYCQQWNSNPPTFGQGTKVEIKRTVAAPSVFIFPPSDEQLKSGTASVVCLLNNFYPREAKVQWKVDNALQSGNSQESVTEQDSKDSTYSLSSTLTLSKADYEKHKVYACEVTHQGLSSPVTKSFNRGEC

SEQ ID NO: 5 - protein, 5 aa, synthetic construct
SYAMS

SEQ ID NO: 6 - protein, 17 aa, synthetic construct
AINSNGGSTYYADSVKG

SEQ ID NO: 7 - protein, 10 aa, synthetic construct
NEEFRRGLAY

SEQ ID NO: 8 - protein, 119 aa, synthetic construct
EVQLVESGGGLVQPGGSLRLSCAASGFTFSSYAMSWVRQAPGKGLELVAAINSNGGSTYYADSVKGRFTISRDNAKNTLYLQMSSLRAEDTAVYYCTRNEEFRRGLAYWGQGTLVTVSS

SEQ ID NO: 9 - protein, 11 aa, synthetic construct
RASENIYSNLA

SEQ ID NO: 10 - protein, 7 aa, synthetic construct
AASNLQS

SEQ ID NO: 11 - protein, 10 aa, synthetic construct
QHFWGTPPWT

SEQ ID NO: 12 - protein, 108 aa, synthetic construct
DIQMTQSPSSLSASVGDRVTITCRASENIYSNLAWYQQKPGKAPKLLIYAASNLQSGVPSRFSGSGSGTDYTLTISSLQPEDFATYYCQHFWGTPPWTFGQGTKLEIK

SEQ ID NO: 13 - protein, 5 aa, synthetic construct
NYVMH

SEQ ID NO: 14 - protein, 17 aa, synthetic construct
YINPYNDDVKYNEKFKG

SEQ ID NO: 15 - protein, 13 aa, synthetic construct
WGYYGSPLYYFDY

SEQ ID NO: 16 - protein, 122 aa, synthetic construct
QVQLVQSGAEVKKPGSSVKVSCKASGYTFTNYVMHWVRQAPGQGLEWMGYINPYNDDVKYNEKFKGRVTITADESTSTAYMELSSLRSEDTAVYYCARWGYYGSPLYYFDYWGQGTLVTVSS

SEQ ID NO: 17 - protein, 10 aa, synthetic construct
RASSRLIYMH

SEQ ID NO: 18 - protein, 7 aa, synthetic construct
ATSNLAS

SEQ ID NO: 19 - protein, 9 aa, synthetic construct
QQWNSNPPT

SEQ ID NO: 20 - protein, 106 aa, synthetic construct
EIVLTQSPATLSLSPGERATLSCRASSRLIYMHWYQQKPGQAPRPLIYATSNLASGIPARFSGSGSGTDFTLTISSLEPEDFAVYYCQQWNSNPPTFGQGTKVEIK